European Patent Application EP 4 417 202 A1, published August 21, 2024. Title: Anti-cancer Action of BAG1-Selective Imidazopyridine Compounds in Steroid Hormone Receptor-Positive Breast and Prostate Cancer. Applicant: Karlsruher Institut für Technologie. Application EP. The sequence listing filed with the application follows.

SEQUENCE LISTING (41 sequences)

SEQ ID NO: 1 - RNA, 21 nt, synthetic construct
  source 1..21: mol_type = other RNA
ggtgcgctcctggacgtagcc

SEQ ID NO: 2 - DNA, 20 bp, synthetic construct
  source 1..20: mol_type = other DNA
ctcctgagcgcaagtactcc

SEQ ID NO: 3 - DNA, 21 bp, synthetic construct
  source 1..21: mol_type = other DNA
gtcaccttcaccgttgttcca

SEQ ID NO: 4 - DNA, 20 bp, synthetic construct
  source 1..20: mol_type = other DNA
cccggttgtcttcctcaccc

SEQ ID NO: 5 - DNA, 20 bp, synthetic construct
  source 1..20: mol_type = other DNA
gcctcccacaatccgagaca

SEQ ID NO: 6 - DNA, 21 bp, synthetic construct
  source 1..21: mol_type = other DNA
tccaggccgagaatacaccta

SEQ ID NO: 7 - DNA, 23 bp, synthetic construct
  source 1..23: mol_type = other DNA
cgatttgcttgtcaaacgtcttc

SEQ ID NO: 8 - DNA, 20 bp, synthetic construct
  source 1..20: mol_type = other DNA
gtgctccctctgttgttcgt

SEQ ID NO: 9 - DNA, 21 bp, synthetic construct
  source 1..21: mol_type = other DNA
gcttctcagacacgatgctct

SEQ ID NO: 10 - DNA, 20 bp, synthetic construct
  source 1..20: mol_type = other DNA
atgggcagcctgatgtctct

SEQ ID NO: 11 - DNA, 18 bp, synthetic construct
  source 1..18: mol_type = other DNA
ggcgccatgcttctcttg

SEQ ID NO: 12 - DNA, 20 bp, synthetic construct
  source 1..20: mol_type = other DNA
gccgactggtgtttatccgt

SEQ ID NO: 13 - DNA, 20 bp, synthetic construct
  source 1..20: mol_type = other DNA
tttcttccctttgcggacca

SEQ ID NO: 14 - DNA, 21 bp, synthetic construct
  source 1..21: mol_type = other DNA
ttcaagggaggcaaatacatg

SEQ ID NO: 15 - DNA, 19 bp, synthetic construct
  source 1..19: mol_type = other DNA
tccaagggccttgtcacag

SEQ ID NO: 16 - DNA, 20 bp, synthetic construct
  source 1..20: mol_type = other DNA
atgcagtggcagtgaccttt

SEQ ID NO: 17 - DNA, 20 bp, synthetic construct
  source 1..20: mol_type = other DNA
catggagccaaagcaggaga

SEQ ID NO: 18 - DNA, 18 bp, synthetic construct
  source 1..18: mol_type = other DNA
agaagaagcgaagaggtc

SEQ ID NO: 19 - DNA, 18 bp, synthetic construct
  source 1..18: mol_type = other DNA
cggacacaaagttatgcc

SEQ ID NO: 20 - DNA, 20 bp, synthetic construct
  source 1..20: mol_type = other DNA
tgcgtgtttgtgcctgtcct

SEQ ID NO: 21 - DNA, 20 bp, synthetic construct
  source 1..20: mol_type = other DNA
gtgctcgcttagtgctccct

SEQ ID NO: 22 - DNA, 20 bp, synthetic construct
  source 1..20: mol_type = other DNA
gactctcagggtcgaaaacg

SEQ ID NO: 23 - DNA, 20 bp, synthetic construct
  source 1..20: mol_type = other DNA
gcggattagggcttcctctt

SEQ ID NO: 24 - DNA, 20 bp, synthetic construct
  source 1..20: mol_type = other DNA
ctcaacgtcgaccccgataa

SEQ ID NO: 25 - DNA, 20 bp, synthetic construct
  source 1..20: mol_type = other DNA
gcctggatcagggtgaagtg

SEQ ID NO: 26 - DNA, 21 bp, synthetic construct
  source 1..21: mol_type = other DNA
gacctcaacgcacagtacgag

SEQ ID NO: 27 - DNA, 22 bp, synthetic construct
  source 1..22: mol_type = other DNA
aggagtcccatgatgagattgt

SEQ ID NO: 28 - DNA, 24 bp, synthetic construct
  source 1..24: mol_type = other DNA
acaccaagtgcaaagaggaaggat

SEQ ID NO: 29 - DNA, 25 bp, synthetic construct
  source 1..25: mol_type = other DNA
gaccaagctttggatttcatttctg

SEQ ID NO: 30 - DNA, 20 bp, synthetic construct
  source 1..20: mol_type = other DNA
cttaatcaactaggcgagag

SEQ ID NO: 31 - DNA, 20 bp, synthetic construct
  source 1..20: mol_type = other DNA
aagctcatccaagaatactg

SEQ ID NO: 32 - DNA, 20 bp, synthetic construct
  source 1..20: mol_type = other DNA
caatggccaccatggagaac

SEQ ID NO: 33 - DNA, 20 bp, synthetic construct
  source 1..20: mol_type = other DNA
aacggtgtcgtcgaaacagc

SEQ ID NO: 34 - DNA, 19 bp, synthetic construct
  source 1..19: mol_type = other DNA
gagtgacaatgaggaagag

SEQ ID NO: 35 - DNA, 20 bp, synthetic construct
  source 1..20: mol_type = other DNA
ctcgttggaaatggagacaa

SEQ ID NO: 36 - DNA, 20 bp, synthetic construct
  source 1..20: mol_type = other DNA
tgagatgtcttcagggagtg

SEQ ID NO: 37 - DNA, 20 bp, synthetic construct
  source 1..20: mol_type = other DNA
agccaggtatttgtggttcg

SEQ ID NO: 38 - DNA, 25 bp, synthetic construct
  source 1..25: mol_type = other DNA
gaccaagctttggatttcatttctg

SEQ ID NO: 39 - DNA, 22 bp, synthetic construct
  source 1..22: mol_type = other DNA
caggttcgtaagcatagagacg

SEQ ID NO: 40 - DNA, 20 bp, synthetic construct
  source 1..20: mol_type = other DNA
gcaggctcagaacagaaagg

SEQ ID NO: 41 - DNA, 20 bp, synthetic construct
  source 1..20: mol_type = other DNA
tccagggtttccacagactc